European Patent Application EP 4 450 649 A1, published October 23, 2024. Title: METHOD AND SYSTEMFOR RISK ASSESSMENTOF AUTISM SPECTRUMDISORDER IN ASUBJECT. Applicant: Tata Consultancy Services Limited. Application EP. The sequence listing filed with the application follows.

SEQUENCE LISTING (9 sequences)

SEQ ID NO: 1 - RNA, 1434 nt, Mogibacterium sp.
  source 1..1434: mol_type = rRNA
gatgaacgctggcggcgtgcctaatacatgcaagtcgagcgagaagcttggaaatgacgcttcggttgaatttccaagcggacagcggcggacgggtgagtaacgcgtaggcaacctgcccctgtacagagggatagccattggaaacgatgattaaaacctcatgacaccgtagtagcacatgctacatcggtcaaagatttatcggtcagggatgggcctccgtctgattaactggttggtgaggtaacggctcaccaaggtgacgatcagtagccgacctgagagggtgatcggccacattggaactgagacacggtccaaacttctacggaaggcagcagtagggaatcttgcacaatgggcgtaagcctgatgcagcaacgccgcgtgaaggatgaaggcttcgggttgtaaacttctgttctaagggaagaaagaaatgacggtaccttaggagcaagccccggctaactacgtgccagcagccgcggtaatacgtagggggcaagcgttatccggaattattgggcgtaaagagtgcgtaggtggttacctaagcgcaaggtttaaattagaggctcaacctctacatgccttgcgaactgggctacttgagtgcaggaggggaaagcggaattcctagtgtagcggtgaaatgcgtagatattaggaggaacaccggcggcgaaggcggctttctggactgtaactgacactgaggcacgaaagcgtgggtagcaaacaggattagataccctggtagtccacgccgtaaacgatgagcactaggtgttgggtccgttaggactcagtgccgcagttaacgcaataagtgtccgcctgggagtacgctcgcaagagtaaactcaaggaattgacgggcacccgcacaagcaggggagcttgtggtttaattcgaagcaacgcgaagaaccttaccagggcttgacatcctgctgacagaaccttaatcggttttttcttcggacagcagagacaggtggtgcatggttgtcgtcagctcgtgtcgtgagatgttgggttaagtcccgcaacgagcgcaacccttgtcgctagttactaacattcagttgaggactctagcgagactgccgaggtcaactcggaggaaggtggggatgacgtcaaatcatcatgccccttatgttctgggctacacacgtgctacaatggtcggtacaatgagatgcaatactgcgaagtggagcgaaacaccaaaaccgatcccagttcggattgtaggctgcaactcgcctacatgaagtcggagttgctagtaatcgcagatcagaatgctgcggtgaatgcgttcccgggtcttgtacacaccgcccgtcacaccatggaagttgggggtgcccaaagtcggttaattaatctatcgcctaaggcaaaaccaatgactggggt

SEQ ID NO: 2 - RNA, 1406 nt, Eubacterium sp.
  source 1..1406: mol_type = rRNA
gtgctgcagagaagagtttgatcctggctcaggatgaacgctggcggcgtgcctaacacatgcaagttgagcgagaaatcacttaaagaagcttcggtagacttaagagatggagagcagcggacgggtgaggaacgcgtgggaaacctgcccttgacaggaggatagccgagagaaatttcgatttaatacttcataaagcagagcattcgcatggatgaactgccaaagaattatcggtcaaggatggtccagcgtctgattagctggttggtaaggtaccggcttaccaaggcgacgatcagtagccggcctgagagggtgaacggccacattggaactgagacacggtccagactctacgggaggcagcagtggggaatattgcacaatgggcgaagcctgatgcagcaacgccgcgtgaaggaagaaggctttcgagtcgtaaacttctgtccaaagggaagaataatgacggtacctttgaagaaagccccggctaactacgtgccagcagccgcggtaatacgtagggggcgagcgttatccggaattactgggcgtaaagagtatgtaggtggttaagtaagcgtagggtttaaggcgacagcccaactgtcgtatgccccgcgagctgtttaacttgagtacaggaggggaaggcggaattcctagtgtagcgctgaaatgcgtagatattaggaggaacaccagtggcgaaggcggccttctggactgtaactgacactgagatacgaaagcgtgggtagcaaacaggattagataccctggtagtccacgccgtaaacgatgagcactaggtgtcgggctcgcaagagttcggtgccggagcaaacgcattaagtgctccgcctggggagtacgcacgcaagtgtgaaactcaaaggaattgacggggacccgcacaagcagcggagcatgtggtttaattcgaagcaacgcgaagaaccttaccaggacttgacatcccactgaaagctcggttaaaactgagcccttcttcggaacagtggagacaggtggtgcatggttgtcgtcagctcgtgtcgtgagatgttgggttaagtcccgcaacgagcgcaacccttgccgttagttgccatcattaagttgggcactctaatgggactgccggggagaacccggaggaaggcggggatgacgtcaaatcatcatgccccttatgttctgggctacacacgtgctacaatggccgtcacagagggaagcgagagagcgatcttaagcgaaaccaaaaaggcggtcccagttcggactgcaggctgcaactcgcctgcacgaagccggagttgctagtaatcgcggatcagaatgtcgcggtgaatgcgttcccgggtcttgtacacaccgccggtggatccgtg

SEQ ID NO: 3 - RNA, 1504 nt, Dialister sp.
  source 1..1504: mol_type = rRNA
cgaacgctggcggcgtgcttaacacatgcaagtcgaacggaaagagatgaaagagcttgctcttttattaatttcagtggcaaacgggtgagtaacacgtaaacaacctgccttaaggatggggataacagacggaaacgactgctaataccgaatacgttctaagcatcgcatggtgcatagaagaaagggtggcctctacaagaaagctatcgccttaagaggggtttgcgactgattaggtagttggtgaggtaacggctcaccaagccgacgatcagtagccggtctgagaggatgaacggccacactggaactgagacacggtccagactcctacgggaggcagcagtggggaatcttccgcaatggacgaaagtctgacggagcaacgccgcgtgaacgaagaaggtcttcggattgtaaagttctgtgattcgggacgaaagggtttgtggtgaataatcattgacattgacggtaccgaaaaagcaagccacggctaactacgtgccagcagccgcggtaatacgtaggtggcaagcgttgtccggaattattgggcgtaaagcgcgcgcaggcggtttcttaagtccatcttaaaagcgtggggctcaaccccatgaggggatggaaactgggaagctggagtatcggagaggaaagtggaattcctagtgtagcggtgaaatgcgtagagattaggaagaacaccggtggcgaaggcgactttctagacgaaaactgacgctgaggcgcgaaagcgtggggagcaaacaggattagataccctggtagtccacgccgtaaacgatggatactaggtgtaggaggtatcgacccctcctgtgccggagttaacgcaataagtatcccgcctgggaagtacgatcgcaagattaaaactcaaaggaattgacgggggcccgcacaagcggtggagtatgtggtttaattcgacgcaacgcgaagaaccttaccaagccttgacattgatcgcaatccatagaaatatggagttcttcttcggaagacgagaaaacaggtggtgcacggctgtcgtcagctcgtgtcgtgagatgttgggttaagtcccgcaacgagcgcaacccctatttcctgttaccagcacgtaaaggtggggactcaggagagaccgccgcggacaacgcggaggaaggcggggatgacgtcaagtcatcatgccccttatggcttgggctacacacgtactacaatgggtgccaacaaagagaagcgaaatcgcgagatggagcggacctcataaacgcacccccagttcagattgcaggctgcaactcgcctgcatgaagtaggaatcgctagtaatcgcgggtcagcataccgcggtgaatacgttcccgggccttgtacacaccgcccgtcacactatgagagttagagacacccgaagccggtgaggtaaccgcaagggaccagccgtctaaggtggagctgatgattggagtgaagtcgtaacaag

SEQ ID NO: 4 - RNA, 1517 nt, Enterococcus sp.
  source 1..1517: mol_type = rRNA
agagtttgatcctggctcaggacgaacgctggcggcgtgcctaatacatgcaagtcgaacgcttctttcctcccgagtgcttgcactcaattggaaagaggagtggcggacgggtgagtaacacgtgggtaacctacccatcagagggggataacacttggaaacaggtgctaataccgcataacagtttatgccgcatggcataagagtgaaaggcgctttcgggtgtcgctgatggatggacccgcggtgcattagctagttggtgaggtaacggctcaccaaggccacgatgcatagccgacctgagagggtgatcggccacactgggactgagacacggcccagactctacgggaggcagcagtagggaatcttcggcaatggacgaaagtctgaccgagcaacgccgcgtgagtgaagaaggttttcggatcgtaaaactctgttgttagagaagaacaaggacgttagtaactgaacgtcccctgacggtatctaaccagaaagccacggctaactacgtgccagcagccgcggtaatacgtaggtggcaagcgttgtccggatttattgggcgtaaagcgagcgcaggcggtttcttaagtctgatgtgaaagcccccggctcaaccggggagggtcattggaaactgggagacttgagtgcagaagaggagagtggaattccatgtgtagcggtgaaatgcgtagatatatggaggaacaccagtggcgaaggcggctctctggtctgtaactgacgctgaggctcgaaagcgtggggagcaaacaggattagataccctggtagtccacgccgtaaacgatgagtgctaagtgttggagggtttccgcccttcagtgctgcagcaaacgcattaagcactccgcctggggagtacgaccgcaaggttgaaactcaaaggaattgacgggggcccgacaagcggtggagcatgtgtttaattcgaagcaacgcgaagaaccttaccaggtcttgacatcctttgaccactctagagatagagctttcccttcggggacaaagtgacagtggtgcatggttgtcgtcagctcgtgtcgtgagatgttgggttaagtccgcaacgagcgcaacccttattgttagttgccatcatttagttgggcactctagcgagactgccggtgacaaaccggaggaaggtggggatgacgtcaaatcatcatgccccttatgacctgggctacacacgtgctacaatgggaagtacaacgagtcgctagaccgcgaggtcatgcaaatctcttaaagcttctctcagttcggattgcaggctgcaactcgcctgcatgaagccggaatcgctagtaatcgcggatcagcacgccgcggtgaatacgttcccgggccttgtacacaccgcccgtcacaccacgagagtttgtaacacccgaagtcggtgaggtaacctttttggagccagccgcctaaggtgggatagatgatttgggtgaagtcgtaacaaggtaacc

SEQ ID NO: 5 - RNA, 1408 nt, Anaeroglobus sp.
  source 1..1408: mol_type = rRNA
cttacgatcgagtggcaaacgggtgagtaacgcgtaaacaacctgccccgcagatggggacaacagctggaaacggctgctaataccgaatacggtcctcttagcgcatggtaagaggaagaaagggtggcctctggaacaagctaccgctgtgggaggggtttgcgtctgattagctggttggaggggtaacggcccaccaaggcgacgatcagtagccggtctgagaggatgaacggccacattggaactgagacacggtccagactcctacgggaggcagcagtggggaatcttccgcaatgggcgaaagcctgacggagcaacgccgcgtgagtgaagacggccttcgggttgtaaagctctgttataggggacgaacggccgggtagcgaagaggtagccggcatgacggtaccgtaagagaaagccacggctaactacgtgccagcagccgcggtaatacgtaggtggcaagcgttgtccggaatgattgggcgtaaagggcgcgcaggcggctgtgtaagtctgtctaaaaagtgcggggctaaaccccgtgagaggatggaaactggacagctgagagtgtcggagaggaaagcggaattcctagtgtagcggtgaaatgcgtagatattaggaggaacaccggtggcgaaagcggctttctggacgacaactgacgctgaggcgcgaaagccaggggagcaaacgggattagataccccggtagtcctggccgtaaacgatgggtactaggtgtaggaggtatcgacccctcctgtgccggagttaacgcaataagtaccccgcctggggagtacggccgcaaggctgaaactcaaaggaattgacgggggcccgcacaagcggtggagtatgtggtttaattcgacgcaacgcgaagaaccttaccaagccttgacattgctcgcaacgggtagagatacctggttcttcttcggaagacgagacaacaggtggtgcacggctgtcgtcagctcgtgtcgtgagatgttgggttaagtcccgcaacgagcgcaacccctatcttcagttaccagcacgtagcggtggggactcaggagagacagccgcagacaatgcggaggaaggcggggacgacgtcaagtcatcatgccccttatggcttgggctacacacgtactacaatggctctaaatagagggaagcgaaggagcgatccggagcaaaccccgcaaacagagtcccagttcggattgcaggctgcaactcgcctgcatgaaggaggaatcgctagtaatcgcaggtcagcatactgcggtgaatacgttcccgggccttgtacacaccgcccgtcacaccacgaaagtcattcacacccgaagccggtgaggtaaccgcaaggagccagccgtcaaaggtg

SEQ ID NO: 6 - RNA, 1465 nt, Peptostreptococcus sp.
  source 1..1465: mol_type = rRNA
gatgaacgctggcggcgtgcctaacacatgcaagtcgagcgagggtttgctcagtattgagtattctaagactagaatgttcaattctgagcaaaaccaagcggcggacgggtgagtaacgcgtgggtaacctgccctatacacatggataacatactgaaaagtttactaatacatgataatatatatttgcggcatcgcagatatatcaaagtgttagcggtataggatggacccgcgtctgattagctagttggtgagataactgcccaccaaggcgacgatcagtagccgacctgagagggtgatcggccacattggaactgagacacggtccaaactcctacgggaggcagcagtggggaatattgcacaatgggcgaaagcctgatgcagcaacgccgcgtgaacgatgaaggtcttcggatcgtaaagttctgttgcaggggaagataatgacggtaccctgtgaggaagccccggctaactacgtgccagcagccgcggtaatacgtagggggctagcgttatccggatttactgggcgtaaagggtgcgtaggtggtccttcaagtcggtggttaaaggctacggctcaaccgtagtaagccgccgaaactggaggacttgagtgcaggagaggaaagtggaattcccagtgtagcggtgaaatgcgtagatattgggaggaacaccagtagcgaaggcggctttctggactgcaactgacactgaggcacgaaagcgtgggtagcaaacaggattagataccctggtagtccacgctgtaaacgatgagtactaggtgtcgggggttacccccctcggtgccgcagctaacgcattaagtactccgcctggggagtacgcacgcaagtgtgaaactcaaaggaattgacggggacccgcacaagtagcggagcatgtggtttaattcgaagcaacgcgaagaaccttacctaagcttgacatccctcggacaggtgtttaatcacacccttccttcgggactgaggtgacaggtggtgcatggttgtcgtcagctcgtgtcgtgagatgttgggttaagtcccgcaacgagcgcaacccttgtctttagttgccagcattcagttgggcactctagagagactgccagggataacctggaggaaggtggggatgacgtcaaatcatcatgccccttatgcttagggctacacacgtgctacaatgggtggtacagagggttgccaaaccgtgaggtggagccaatcccttaaagccattctcagttcggattgtaggctgaaactcgcctacatgaagctggagttactagtaatcgcagatcagaatgctgcggtgaatgcgttcccgggtcttgtacacaccgcccgtcacaccacgggagtcggaaacacccgaagccgattatccaaccgcaaggaggaagtcgtcgaaggtggcgtcnataactggggtg

SEQ ID NO: 7 - RNA, 1487 nt, Solobacterium sp.
  source 1..1487: mol_type = rRNA
agagtttgatcctggctcagtatgaactctgccggcgtgcctaatacttgcaagtcgaacgctgaagatctagcttgctagatcgaaggagtgccgaacgggtgagtaatacataagcaacctacccacgaagactgggataatctctggaaacggggactaataccggataggtaatcggaaggcatcttctggttattaaaggttaaaaacactggtggatgggcttatggcgcattagttagttggtgaggtaacggcccaccaagacgatgatgcgtagccggcctgagagggtgaacggccacattgggactgagacacggcccagactctacgggaggcagcagtagggaattttcggcaataggggcaaccctgaccgagcaacgccgcgtgagtgaagacggccttcgggttgtaaaagctcttgtttgtaagggaagaacggtagatagagaatatctaagtgacggtaccttaccagaaagccacggctaactacgtgccagcagccgcggtaatacgtaggtggcgaccgttatccggaattattggccgtaaagggtgcgtaggcggcctgttaagtaagtggttaaattgttgggctcaacccaatccagccacttaaactggcaggctagagtattggagaggcaagtggaattccatgtgtagcggtaaaatgcgtagatatatggaggaacaccagtggcgaaggcggcttgctagccaaagactgacgctcatgcacgaaaccgtggggagccaataggattagataccctagtagtccacgccgtaaccgatgaatactaagtattggggaaactcagtgctgcactaacgcaataagtattccgcctgtggagtatgcacgcaagtgtgaaacataaaggaattgacgggggcccgcacaagcggtggagtatgtggtttaattcgacgcaacgcgaagaaccttaccaggccttgacatcccttgcaaagctgtagagatacagtagaggttatcaaggagacaggtggttgcatggtgtcgtcagctcgtgtcgtgagatgttgggttaagtccggcaacgagcgcaacccttgccttcagttaccagcatttagttggggactctggagggactgccggtgataaaccggaggaaggtggggatgacgtcaaatcatcatgccccttatggcctgggctacacacgtactacaatggctgttacaacgtgcagcgacctagcgataggaagcgaatcactaaaagacagtctcagttcggattgaagtctgcaactcgacttcatgaagctggaatcgctagtaatcgcggatcagaatgccgcggtgaatacgttctcgggccttgtacacaccgcccgtcataccatgagagctggtaatacccgaggccggtggcctaaccgcaaggaaggagccgtcgaaggtaggactagtgattggggtcaagtcgtaacaaggtaacc

SEQ ID NO: 8 - RNA, 1450 nt, Actinomyces sp.
  source 1..1450: mol_type = rRNA
tcctgactcaggacgaacgctgccggcgtacataacacatgcaagtcgaacggtgaaggggcctgcttttgtgggtcctggatgagtggcgaacgggtgagtaacacgtgagtaacctgcccccttcttctggataaccgcatgaaagtgtggctaatacgggatattctgggtctgtcgcatggtgggcctgggaaagattgcgccttttttggtgtttttggtgggggatgggctcgcggcctatcagcttgttggtggggtgatggcctgccaaggcggtgacgggtagccggcctgagagggtggacggtcacactgggactgagacacggcccagactcctacgggaggcagcagtggggaatattgcacaatgggcgcaagcctgatgcagcgacgccgcgtgagggatggaggccttcgggttgtgaacctctttcgccagtgaagcaggcctgcctcgtttgtgggtgggttgacggtagctggataagaagcgccggctaactacgtgccagcagccgcggtaatacgtagggcgcgagcgttgtccggaattattgggcgtaaagagctcgtaggcggctggtcgcgtctgtcgtgaaatcctctggcttaactgggggcttgcggtgggtacgggccggcttgagtgcggtaggggagactggaactcctggtgtagcggtggaatgcgcagatatcaggaagaacaccggtggcgaaggcgggtctctgggccgttactgacgctgaggagcgaaagcgtggggagcgaacaggattagataccctggtagtccacgccgtaaacgttgggcactaggtgtggggggccttttccgggtcttccgcgccgtagctaacgcattaagtgccccgcctggggagtacggccgcaaggctaaaactcaaaggaattgacgggggcccgcacaagcggcggagcatgcggattaattcgatgcaacgcgaagaaccttaccaaggcttgacatgtgccggtctgctccggagacggggtttcctcctttgtgggggctggttcacaggtggtgcatggttgtcgtcagctcgtgtcgtgagatgttgggttaagtcccgcaacgagcgcaacccttgtctcgtgttgccagcacgttgtggtggggactcgcgggagactgccggggtcaactcggaggaaggtggggatgacgtcaaatcatcatgccccttatgtcttgggcttcacgcatgctacaatggccggtacagagggctgcgataccgtgaggtggagcgaatcccttaaagccggtctcagttcggatcggtgtctgcaactcgacaccgtgaagttggagtcgctagtaatcgcagatcagcaacgctgcggtgaatacgttctcgggccttgtacacaccgcccgtcacgtcatgaaagtcggcaacacccgaagcccgt

SEQ ID NO: 9 - RNA, 1446 nt, Alistipes sp.
  source 1..1446: mol_type = rRNA
gatgaacgctagcggcaggcttaacacatgcaagtcgaggggcagcacgaggtagcaatactttggtggcgaccggcgcacgggtgcgtaacgcgtatgcaacctacctttaacaggggcataacactgagaaattggtactaattccccataacattcgagaaggcatcttcttgggttaaaaactccggtggttaaagatgggcatgcgttgtattagctagttggtgaggtaacggctcaccaaggcaacgatacatagggggactgagaggttaaccccccacattggtactgagacacggaccaaactcctacgggaggcagcagtgaggaatattggtcaatggacgcaagtctgaaccagccatgccgcgtgcaggaagacggctctatgagttgtaaactgcttttgtactagggtaaacgctcttacgtgtaggagcctgaaagtatagtacgaataaggatcggctaactccgtgccagcagccgcggtaatacggaggatccaagcgttatccggatttattgggtttaaagggtgcgtaggcggtttgataagttagaggtgaaataccggggctcaactccggaactgcctctaatactgttgaactagagagtagttgcggtaggcggaatgtatggtgtagcggtgaaatgcttagagatcatacagaacaccgattgcgaaggcagcttaccaaactatatctgacgttgaggcacgaaagcgtggggagcaaacaggattagataccctggtagtccacgcagtaaacgatgataactcgttgtcggcgatacacagtcggtgactaagcgaaagcgataagttatccacctggggagtacgttcgcaagaatgaaactcaaaggaattgacgggggcccgcacaagcggaggaacatgtggtttaattcgatgatacgcgaggaaccttacccgggcttgaaagttagtgacgattctggaaacaggatttcccttcggggcacgaaactaggtgctgcatggttgtcgtcagctcgtgccgtgaggtgtcgggttaagtcccataacgagcgcaacccctaccgttagttgccatcaggtcaagctgggcactctggcgggactgccggtgtaagccgagaggaaggtggggatgacgtcaaatcagcacggcccttacgtccggggctacacacgtgttacaatggtaggtacagagggccgctaccccgcgaggggatgccaatctcgaaagcctatctcagttcggatcggaggctgaaacccgcctccgtgaagttggattcgctagtaatcgcgcatcagccatggcgcggtgaatacgttcccgggccttgtacacaccgcccgtcaagccatggaagctgggggtgcctgaagttcgtgaccgcaaggagcgacctagggcaaaaccggtgactggggct